European Patent Application EP 4 238 987 A1, published September 6, 2023. Title: Modified Signal Peptide. Applicant: Kao Corporation. The sequence listing filed with the application follows.

SEQUENCE LISTING (84 sequences)

SEQ ID NO: 1 - protein, 24 aa, Bacillus sp.
  YoaW_signal
MKKMLMLAFTFLLALTIHVGEASA

SEQ ID NO: 2 - protein, 32 aa, Bacillus sp.
  lipA_signal
MKFVKRRIIALVTILMLSVTSLFALQPSAKAA

SEQ ID NO: 3 - protein, 24 aa, Bacillus sp.
  pelB_signal
MKRLCLWFTVFSLFLVLLPGKALG

SEQ ID NO: 4 - protein, 42 aa, Bacillus sp.
  YncM_signal
MAKPLSKGGILVKKVLIAGAVGTAVLFGTLSSGIPGLPAADA

SEQ ID NO: 5 - protein, 29 aa, Bacillus sp.
  S237_signal
MLRKKTKQLISSILILVLLLSLFPAALAA

SEQ ID NO: 6 - protein, 31 aa, Bacillus sp.
  AmyQ_signal
MIQKRKRTVSFRLVLMCTLLFVSLPITKTSA

SEQ ID NO: 7 - protein, 16 aa, Bacillus sp.
  N-side region of YoaW_signal
MKKMLMLAFTFLLALT

SEQ ID NO: 8 - protein, 26 aa, Bacillus sp.
  N-side region of lipA_signal
MKFVKRRIIALVTILMLSVTSLFALQ

SEQ ID NO: 9 - protein, 18 aa, Bacillus sp.
  N-side region of pelB_signal
MKRLCLWFTVFSLFLVLL

SEQ ID NO: 10 - protein, 34 aa, Bacillus sp.
  N-side region of YncM_signal
MAKPLSKGGILVKKVLIAGAVGTAVLFGTLSSGI

SEQ ID NO: 11 - protein, 23 aa, Bacillus sp.
  N-side region of S237_signal
MLRKKTKQLISSILILVLLLSLF

SEQ ID NO: 12 - protein, 24 aa, Bacillus sp.
  N-side region of AmyQ_signal
MIQKRKRTVSFRLVLMCTLLFVSL

SEQ ID NO: 13 - protein, 6 aa, Artificial
  C-terminal region of modified signal peptide
GGAAFA

SEQ ID NO: 14 - protein, 6 aa, Artificial
  C-terminal region of modified signal peptide
AGPASA

SEQ ID NO: 15 - protein, 6 aa, Artificial
  C-terminal region of modified signal peptide
GGSASA

SEQ ID NO: 16 - protein, 6 aa, Artificial
  C-terminal region of modified signal peptide
GGAASA

SEQ ID NO: 17 - protein, 6 aa, Artificial
  C-terminal region of modified signal peptide
GGSAFA

SEQ ID NO: 18 - protein, 6 aa, Artificial
  C-terminal region of modified signal peptide
GGAAHA

SEQ ID NO: 19 - protein, 6 aa, Artificial
  C-terminal region of modified signal peptide
AGSAFA

SEQ ID NO: 20 - protein, 6 aa, Artificial
  C-terminal region of modified signal peptide
AGPAFA

SEQ ID NO: 21 - protein, 6 aa, Artificial
  C-terminal region of modified signal peptide
AGSAHA

SEQ ID NO: 22 - protein, 6 aa, Artificial
  C-terminal region of modified signal peptide
PGSAFA

SEQ ID NO: 23 - protein, 6 aa, Artificial
  C-terminal region of modified signal peptide
GGSAHA

SEQ ID NO: 24 - protein, 6 aa, Artificial
  C-terminal region of modified signal peptide
PGAAFA

SEQ ID NO: 25 - protein, 6 aa, Artificial
  C-terminal region of modified signal peptide
PGSASA

SEQ ID NO: 26 - protein, 6 aa, Artificial
  C-terminal region of modified signal peptide
AGSASA

SEQ ID NO: 27 - protein, 6 aa, Artificial
  C-terminal region of modified signal peptide
AGPAHA

SEQ ID NO: 28 - protein, 6 aa, Artificial
  C-terminal region of modified signal peptide
PGSAHA

SEQ ID NO: 29 - protein, 6 aa, Artificial
  C-terminal region of modified signal peptide
PGAAHA

SEQ ID NO: 30 - protein, 6 aa, Artificial
  C-terminal region of modified signal peptide
PGAASA

SEQ ID NO: 31 - protein, 29 aa, Artificial
  Modified signal peptide
MLRKKTKQLISSILILVLLLSLFPGSASA

SEQ ID NO: 32 - protein, 29 aa, Artificial
  Modified signal peptide
MLRKKTKQLISSILILVLLLSLFAGSASA

SEQ ID NO: 33 - protein, 29 aa, Artificial
  Modified signal peptide
MLRKKTKQLISSILILVLLLSLFAGPAHA

SEQ ID NO: 34 - protein, 29 aa, Artificial
  Modified signal peptide
MLRKKTKQLISSILILVLLLSLFPGSAHA

SEQ ID NO: 35 - protein, 40 aa, Artificial
  Modified signal peptide
MAKPLSKGGILVKKVLIAGAVGTAVLFGTLSSGIGGSASA

SEQ ID NO: 36 - DNA, 48 bp, Bacillus sp.
  N-side region of YoaW_signal
atgaaaaagatgttgatgttagcttttacatttcttttggctttgact

SEQ ID NO: 37 - DNA, 78 bp, Bacillus sp.
  N-side region of lipA_signal
atgaaatttgtaaaaagaaggatcattgcacttgtaacaattttgatgctgtctgttacatcgctgtttgcgttgcag

SEQ ID NO: 38 - DNA, 54 bp, Bacillus sp.
  N-side region of pelB_signal
atgaaacgactttgtttatggttcaccgtctttagcttgtttttggttctcttg

SEQ ID NO: 39 - DNA, 102 bp, Bacillus sp.
  N-side region of YncM_signal
atggcgaaaccactatcaaaagggggaattttggtgaaaaaagtattgattgcaggtgcagtaggaacagcagttcttttcggaaccctttcatcaggtata

SEQ ID NO: 40 - DNA, 69 bp, Bacillus sp.
  N-side region of S237_signal
atgttaagaaagaaaacaaagcagttgatttcttccattcttattttagttttacttctatctttattt

SEQ ID NO: 41 - DNA, 72 bp, Bacillus sp.
  N-side region of AmyQ_signal
atgattcaaaaacgaaagcggacagtttcgttcagacttgtgcttatgtgcacgctgttatttgtcagtttg

SEQ ID NO: 42 - DNA, 18 bp, Artificial
  C-terminal region of modified signal peptide
ggcggcgcagcatttgca

SEQ ID NO: 43 - DNA, 18 bp, Artificial
  C-terminal region of modified signal peptide
gcaggcccggcatcagca

SEQ ID NO: 44 - DNA, 18 bp, Artificial
  C-terminal region of modified signal peptide
ggcggctcagcatcagca

SEQ ID NO: 45 - DNA, 18 bp, Artificial
  C-terminal region of modified signal peptide
ggcggcgcagcatcagca

SEQ ID NO: 46 - DNA, 18 bp, Artificial
  C-terminal region of modified signal peptide
ggcggctcagcatttgca

SEQ ID NO: 47 - DNA, 18 bp, Artificial
  C-terminal region of modified signal peptide
ggcggcgcagcacatgca

SEQ ID NO: 48 - DNA, 18 bp, Artificial
  C-terminal region of modified signal peptide
gcaggctcagcatttgca

SEQ ID NO: 49 - DNA, 18 bp, Artificial
  C-terminal region of modified signal peptide
gcaggcccggcatttgca

SEQ ID NO: 50 - DNA, 18 bp, Artificial
  C-terminal region of modified signal peptide
gcaggctcagcacatgca

SEQ ID NO: 51 - DNA, 18 bp, Artificial
  C-terminal region of modified signal peptide
ccgggctcagcatttgca

SEQ ID NO: 52 - DNA, 18 bp, Artificial
  C-terminal region of modified signal peptide
ggcggctcagcacatgca

SEQ ID NO: 53 - DNA, 18 bp, Artificial
  C-terminal region of modified signal peptide
ccgggcgcagcatttgca

SEQ ID NO: 54 - DNA, 18 bp, Artificial
  C-terminal region of modified signal peptide
ccgggctcagcatcagca

SEQ ID NO: 55 - DNA, 18 bp, Artificial
  C-terminal region of modified signal peptide
gcaggctcagcatcagca

SEQ ID NO: 56 - DNA, 18 bp, Artificial
  C-terminal region of modified signal peptide
gcaggcccggcacatgca

SEQ ID NO: 57 - DNA, 18 bp, Artificial
  C-terminal region of modified signal peptide
ccgggctcagcacatgca

SEQ ID NO: 58 - DNA, 18 bp, Artificial
  C-terminal region of modified signal peptide
ccgggcgcagcacatgca

SEQ ID NO: 59 - DNA, 18 bp, Artificial
  C-terminal region of modified signal peptide
ccgggcgcagcatcagca

SEQ ID NO: 60 - DNA, 87 bp, Artificial
  Modified signal peptide
atgttaagaaagaaaacaaagcagttgatttcttccattcttattttagttttacttctatctttatttccgggctcagcatcagca

SEQ ID NO: 61 - DNA, 87 bp, Artificial
  Modified signal peptide
atgttaagaaagaaaacaaagcagttgatttcttccattcttattttagttttacttctatctttatttgcaggctcagcatcagca

SEQ ID NO: 62 - DNA, 87 bp, Artificial
  Modified signal peptide
atgttaagaaagaaaacaaagcagttgatttcttccattcttattttagttttacttctatctttatttgcaggcccggcacatgca

SEQ ID NO: 63 - DNA, 87 bp, Artificial
  Modified signal peptide
atgttaagaaagaaaacaaagcagttgatttcttccattcttattttagttttacttctatctttatttccgggctcagcacatgca

SEQ ID NO: 64 - DNA, 120 bp, Artificial
  Modified signal peptide
atggcgaaaccactatcaaaagggggaattttggtgaaaaaagtattgattgcaggtgcagtaggaacagcagttcttttcggaaccctttcatcaggtataggcggctcagcatcagca

SEQ ID NO: 65 - DNA, 575 bp, Bacillus sp. KSM-S237
  KSM-S237 promoter
gatttgccgatgcaacaggcttatatttagaggaaatttctttttaaattgaatacggaataaaatcaggtaaacaggtcctgattttatttttttgagttttttagagaactgaagattgaaataaaagtagaagacaaaggacataagaaaattgcattagttttaattatagaaaacgcctttttataattatttatacctagaacgaaaatactgtttcgaaagcggtttactataaaaccttatattccggctcttttttaaaacagggggtaaaaattcactctagtattctaatttcaacatgctataataaatttgtaagacgcaatatgcatctctttttttacgatatatgtaagcggttaaccttgtgctatatgccgatttaggaaggggggtagattgagtcaagtagtaataatatagataacttataagttgttgagaagcaggagagcatctgggttactcacaagtttttttaaaactttaacgaaagcactttcggtaatgcttatgaatttagctatttgattcaattactttaaaaatatttaggaggtaatatg

SEQ ID NO: 66 - DNA, 617 bp, Bacillus sp. KSM-64
  KSM-64 promoter
gaacaagtacttaccattttagagtcaaaagatagaagccaagcaggatttgccgatgcaaccggcttatatttagagggaatttctttttaaattgaatacggaataaaatcaggtaaacaggtcctgattttatttttttgaatttttttgagaactaaagattgaaatagaagtagaagacaacggacataagaaaattgtattagttttaattatagaaaacgcttttctataattatttatacctagaacgaaaatactgtttcgaaagcggtttactataaaaccttatattccggctctttttttaaacagggggtgaaaattcactctagtattctaatttcaacatgctataataaatttgtaagacgcaatatacatcttttttttatgatatttgtaagcggttaaccttgtgctatatgccgatttaggaagggggtagattgagtcaagtagtcataatttagataacttataagttgttgagaagcaggagagaatctgggttactcacaagttttttaaaacattatcgaaagcactttcggttatgcttatgaatttagctatttgattcaattactttaataattttaggaggtaatatg

SEQ ID NO: 67 - DNA, 193 bp, Bacillus subtilis
  spoVG promoter
taagaaaagtgattctgggagagccgggatcacttttttatttaccttatgcccgaaatgaaagctttatgacctaattgtgtaactatatcctattttttcaaaaaatattttaaaaacgagcaggatttcagaaaaaatcgtggaattgatacactaatgcttttatatagggaaaaggtggtgaactact

SEQ ID NO: 68 - protein, 136 aa, Camelus dromedarius
DVQLVESGGGSVQAGGSLRLSCAASGSTDSIEYMTWFRQAPGKAREGVAALYTHTGNTYYTDSVKGRFTISQDKAKNMAYLRMDSVKSEDTAIYTCGATRKYVPVRFALDQSSYDYWGQGTQVTVSSRGRHHHHHH

SEQ ID NO: 69 - protein, 131 aa, Unknown
  Camelidae
QVQLVESGGGLVQAGGSLRLSCAASGRTFSSYGMGWFRQAPGKEREFVAAIRWNGGSTYYADSVKGRFTISRDNAKNTVYLQMNSLKPEDTAVYYCAAGRWDKYGSSFQDEYDYWGQGTQVTVSSHHHHHH

SEQ ID NO: 70 - DNA, 15 bp, Artificial
gcagctcttgcagca

SEQ ID NO: 71 - DNA, 15 bp, Artificial
tctattaaactagtt

SEQ ID NO: 72 - DNA, 25 bp, Artificial
  Primer
tgctgcaagagctgccggaaataaa

SEQ ID NO: 73 - DNA, 21 bp, Artificial
  Primer
tctattaaactagttataggg

SEQ ID NO: 74 - DNA, 25 bp, Artificial
  Primer
atgatgttaagaaagaaaacaaagc

SEQ ID NO: 75 - DNA, 20 bp, Artificial
  Primer
cccgggaattcctgttataa

SEQ ID NO: 76 - DNA, 35 bp, Artificial
  Primer
acaggaattcccgggtaagaaaagtgattctggga

SEQ ID NO: 77 - DNA, 35 bp, Artificial
  Primer
ctttcttaacatcatagtagttcaccaccttttcc

SEQ ID NO: 78 - DNA, 20 bp, Artificial
  Primer
caagttcaactggttgaatc

SEQ ID NO: 79 - DNA, 20 bp, Artificial
  Primer
agtagttcacctccttttcc

SEQ ID NO: 80 - DNA, 35 bp, Artificial
  Primer
aggaggtgaactactatggcgaaaccactatcaaa

SEQ ID NO: 81 - DNA, 35 bp, Artificial
  Primer
aaccagttgaacttgagcgtctgccgcgggtaaac

SEQ ID NO: 82 - protein, 6 aa, Artificial
  C-terminal region of modified signal peptide
GGPASA

SEQ ID NO: 83 - protein, 6 aa, Artificial
  C-terminal region of modified signal peptide
GGPAHA

SEQ ID NO: 84 - protein, 6 aa, Artificial
  C-terminal region of modified signal peptide
GGPAFA